European Patent Specification EP 4 200 319 B1, published April 16, 2025. Title: Annexin A1 N-terminal peptide formulations and methods. Applicant: ResoTher Pharma Aps. The sequence listing filed with the application follows.

SEQUENCE LISTING (11 sequences)

SEQ ID NO: 1 - protein, 346 aa, Homo sapiens
MAMVSEFLKQAWFIENEEQEYVQTVKSSKGGPGSAVSPYPTFNPSSDVAALHKAIMVKGVDEATIIDILTKRNNAQRQQIKAAYLQETGKPLDETLKKALTGHLEEVVLALLKTPAQFDADELRAAMKGLGTDEDTLIEILASRTNKEIRDINRVYREELKRDLAKDITSDTSGDFRNALLSLAKGDRSEDFGVNEDLADSDARALYEAGERRKGTDVNVFNTILTTRSYPQLRRVFQKYTKYSKHDMNKVLDLELKGDIEKCLTAIVKCATSKPAFFAEKLHQAMKGVGTRHKALIRIMVSRSEIDMNDIKAFYQKMYGISLCQAILDETKGDYEKILVALCGGN

SEQ ID NO: 2 - protein, 54 aa, Homo sapiens
MAMVSEFLKQAWFIENEEQEYVQTVKSSKGGPGSAVSPYPTFNPSSDVAALHKA

SEQ ID NO: 3 - protein, 53 aa, Homo sapiens
AMVSEFLKQAWFIENEEQEYVQTVKSSKGGPGSAVSPYPTFNPSSDVAALHKA

SEQ ID NO: 4 - protein, 49 aa, Homo sapiens
AMVSEFLKQAWFIENEEQEYVQTVKSSKGGPGSAVSPYPTFNPSSDVAA

SEQ ID NO: 5 - protein, 47 aa, Homo sapiens
AMVSEFLKQAWFIENEEQEYVQTVKSSKGGPGSAVSPYPTFNPSSDV

SEQ ID NO: 6 - protein, 45 aa, Homo sapiens
AMVSEFLKQAWFIENEEQEYVQTVKSSKGGPGSAVSPYPTFNPSS

SEQ ID NO: 7 - protein, 49 aa, Artificial sequence
  Mutated Annexin A1 2-50 V24L
  MISC_FEATURE (24)..(24): Amino acid V substituted with L
AMVSEFLKQAWFIENEEQEYVQTLKSSKGGPGSAVSPYPTFNPSSDVAA

SEQ ID NO: 8 - protein, 47 aa, Artificial sequence
  Mutated Annexin A1 2-48 V24L
  MISC_FEATURE (24)..(24): Amino acid V substituted with L
AMVSEFLKQAWFIENEEQEYVQTLKSSKGGPGSAVSPYPTFNPSSDV

SEQ ID NO: 9 - protein, 45 aa, Artificial sequence
  Mutated Annexin A1 2-46 V24L
  MISC_FEATURE (24)..(24): Amino acid V substituted with L
AMVSEFLKQAWFIENEEQEYVQTLKSSKGGPGSAVSPYPTFNPSS

SEQ ID NO: 10 - protein, 25 aa, Homo sapiens
AMVSEFLKQAWFIENEEQEYVQTVK

SEQ ID NO: 11 - protein, 25 aa, Artificial sequence
  Mutated Annexin A1 2-26 V24L
  MISC_FEATURE (24)..(24): Amino acid V substituted with L
AMVSEFLKQAWFIENEEQEYVQTLK